European Patent Application EP 4 458 969 A1, published November 6, 2024. Title: 靶向HIV的siRNA和shRNA及其相应的组合、表达盒、细胞及其应用. Applicant: 北京三诺佳邑生物技术有限责任公司. Application CN. The sequence listing filed with the application follows.

SEQUENCE LISTING (29 sequences)

SEQ ID NO: 1 - RNA, 24 nt, synthetic construct
  misc_feature 1..24: note
  source 1..24: mol_type = other RNA
atcaatgaggaagctgcagaatgg

SEQ ID NO: 2 - RNA, 27 nt, synthetic construct
  misc_feature 1..27: note
  source 1..27: mol_type = other RNA
gggaagtgacatagcaggaactactag

SEQ ID NO: 3 - RNA, 29 nt, synthetic construct
  misc_feature 1..29: note
  source 1..29: mol_type = other RNA
taaataaaatagtaagaatgtatagccct

SEQ ID NO: 4 - RNA, 27 nt, synthetic construct
  misc_feature 1..27: note
  source 1..27: mol_type = other RNA
ggatggtgcttcaagctagtaccagtt

SEQ ID NO: 5 - RNA, 26 nt, synthetic construct
  misc_feature 1..26: note
  source 1..26: mol_type = other RNA
accacacacaaggctacttccctgat

SEQ ID NO: 6 - RNA, 19 nt, synthetic construct
  misc_feature 1..19: note
  source 1..19: mol_type = other RNA
caatgaggaagctgcagaa

SEQ ID NO: 7 - RNA, 19 nt, synthetic construct
  misc_feature 1..19: note
  source 1..19: mol_type = other RNA
gtgacatagcaggaactac

SEQ ID NO: 8 - RNA, 19 nt, synthetic construct
  misc_feature 1..19: note
  source 1..19: mol_type = other RNA
atagtaagaatgtatagcc

SEQ ID NO: 9 - RNA, 19 nt, synthetic construct
  misc_feature 1..19: note
  source 1..19: mol_type = other RNA
tgcttcaagctagtaccag

SEQ ID NO: 10 - RNA, 19 nt, synthetic construct
  misc_feature 1..19: note
  source 1..19: mol_type = other RNA
cacaaggctacttccctga

SEQ ID NO: 11 - DNA, 47 bp, synthetic construct
  misc_feature 1..47: note
  source 1..47: mol_type = other DNA
caatgaggaagctgcagaattcaagagattctgcagcttcctcattg

SEQ ID NO: 12 - DNA, 47 bp, synthetic construct
  misc_feature 1..47: note
  source 1..47: mol_type = other DNA
gtgacatagcaggaactacttcaagagagtagttcctgctatgtcac

SEQ ID NO: 13 - DNA, 47 bp, synthetic construct
  misc_feature 1..47: note
  source 1..47: mol_type = other DNA
atagtaagaatgtatagccttcaagagaggctatacattcttactat

SEQ ID NO: 14 - DNA, 47 bp, synthetic construct
  misc_feature 1..47: note
  source 1..47: mol_type = other DNA
tgcttcaagctagtaccagttcaagagactggtactagcttgaagca

SEQ ID NO: 15 - DNA, 47 bp, synthetic construct
  misc_feature 1..47: note
  source 1..47: mol_type = other DNA
cacaaggctacttccctgattcaagagatcagggaagtagccttgtg

SEQ ID NO: 16 - DNA, 22 bp, synthetic construct
  misc_feature 1..22: note
  source 1..22: mol_type = other DNA
atcgaattcccgtttgtgctag

SEQ ID NO: 17 - DNA, 33 bp, synthetic construct
  misc_feature 1..33: note
  source 1..33: mol_type = other DNA
aagcttgcgggatccccgcggctctaaaattta

SEQ ID NO: 18 - DNA, 21 bp, synthetic construct
  misc_feature 1..21: note
  source 1..21: mol_type = other DNA
agcgcagcgagtcagtgagcg

SEQ ID NO: 19 - DNA, 35 bp, synthetic construct
  misc_feature 1..35: note
  source 1..35: mol_type = other DNA
ggatcccgcaagcttagatccgcactttttaaaag

SEQ ID NO: 20 - RNA, 19 nt, synthetic construct
  misc_feature 1..19: note
  source 1..19: mol_type = other RNA
ttctgcagcttcctcattg

SEQ ID NO: 21 - RNA, 19 nt, synthetic construct
  misc_feature 1..19: note
  source 1..19: mol_type = other RNA
gtagttcctgctatgtcac

SEQ ID NO: 22 - RNA, 19 nt, synthetic construct
  misc_feature 1..19: note
  source 1..19: mol_type = other RNA
ggctatacattcttactat

SEQ ID NO: 23 - RNA, 19 nt, synthetic construct
  misc_feature 1..19: note
  source 1..19: mol_type = other RNA
ctggtactagcttgaagca

SEQ ID NO: 24 - RNA, 19 nt, synthetic construct
  misc_feature 1..19: note
  source 1..19: mol_type = other RNA
tcagggaagtagccttgtg

SEQ ID NO: 25 - RNA, 47 nt, synthetic construct
  misc_feature 1..47: note
  source 1..47: mol_type = other RNA
caatgaggaagctgcagaattcaagagattctgcagcttcctcattg

SEQ ID NO: 26 - RNA, 47 nt, synthetic construct
  misc_feature 1..47: note
  source 1..47: mol_type = other RNA
gtgacatagcaggaactacttcaagagagtagttcctgctatgtcac

SEQ ID NO: 27 - RNA, 47 nt, synthetic construct
  misc_feature 1..47: note
  source 1..47: mol_type = other RNA
atagtaagaatgtatagccttcaagagaggctatacattcttactat

SEQ ID NO: 28 - RNA, 47 nt, synthetic construct
  misc_feature 1..47: note
  source 1..47: mol_type = other RNA
tgcttcaagctagtaccagttcaagagactggtactagcttgaagca

SEQ ID NO: 29 - RNA, 47 nt, synthetic construct
  misc_feature 1..47: note
  source 1..47: mol_type = other RNA
cacaaggctacttccctgattcaagagatcagggaagtagccttgtg